European Patent Application EP 4 248 986 A1, published September 27, 2023. Title: USE OF A POLYPEPTIDE HAVING A SUPEROXIDE DISMUTASE ACTIVITY AND AN EXTRACELLUAR VESICLE FOR TREATING OR PREVENTING A RESPIRATORY VIRAL INFECTION. Applicant: GENOFOCUS CO., LTD. The sequence listing filed with the application follows.

SEQUENCE LISTING (1 sequence)

SEQ ID NO: 1 - protein, 201 aa, Artificial Sequence
  Bacillus amyloliquefaciens
MAYKLPELPYAYDALEPHIDKETMTIHHTKHHNTYVTNLNKAIEGSALAEKSVDELVADLNAVPEDIRTAVRNNGGGHANHSLFWTLLSPNGGGEPTGELAEEIKSTFGSFDQFKEKFAAAAAGRFGSGWAWLVVNNGKLEITSTPNQDSPLSEGKTPVLGLDVWEHAYYLNYQNRRPDYISAFWNVVNWDEVARLYSEAK